European Patent Application EP 4 624 486 A1, published October 1, 2025. Title: 带有修饰结构的多肽及其应用. Applicant: 广东众生睿创生物科技有限公司. The sequence listing filed with the application follows.

SEQUENCE LISTING (43 sequences)

SEQ ID NO: 1 - protein, 39 aa, synthetic construct
  SITE 2: note = X is Aib
  SITE 13: note = L is alpha- Methylleucine
  SITE 20: note = X is Aib
YXQGTFTSDYSILLDKKAQXKFIEYLLEGGPSSGAPPPS

SEQ ID NO: 2 - protein, 39 aa, synthetic construct
  SITE 2: note = X is Aib
  SITE 13: note = L is alpha- Methylleucine
  SITE 20: note = X is Aib
YXQGTFTSDYSILLDKKAQXAFIKWLLKGGPSSGAPPPS

SEQ ID NO: 3 - protein, 39 aa, synthetic construct
  SITE 2: note = X is Aib
  SITE 30: note = X is Aib
  SITE 13: note = L is alpha- Methylleucine
YXQGTFTSDYSILLDKKAQXAFIEKLLEGGPSSGAPPPS

SEQ ID NO: 4 - protein, 39 aa, synthetic construct
  SITE 2: note = X is Aib
  SITE 20: note = X is Aib
HXHGTFTSDYSIYLEKKYAXEFVKWLLKGGPSSGAPPPS

SEQ ID NO: 5 - protein, 39 aa, synthetic construct
  SITE 2: note = X is Aib
  SITE 20: note = X is Aib
HXHGTFTSDYSIYLEKKYAXKFVQWLLEGGPSSGAPPPS

SEQ ID NO: 6 - protein, 39 aa, synthetic construct
  SITE 2: note = X is Aib
  SITE 20: note = X is Aib
  SITE 13: note = L is alpha- Methylleucine
YXQGTFTSDYSILLDKKAQXAFIQKLLKGGPSSGAPPPS

SEQ ID NO: 7 - protein, 39 aa, synthetic construct
  SITE 2: note = X is Aib
  SITE 20: note = X is Aib
  SITE 13: note = L is alpha- Methylleucine
YXQGTFTSDYSILLDKQAQXAFIEKLLKGGPSSGAPPPS

SEQ ID NO: 8 - protein, 39 aa, synthetic construct
  SITE 2: note = X is Aib
  SITE 20: note = X is Aib
  SITE 13: note = L is alpha- Methylleucine
YXQGTFTSDYSILLDKEAQXAFIEKLLKGGPSSGAPPPS

SEQ ID NO: 9 - protein, 39 aa, synthetic construct
  SITE 2: note = X is Aib
  SITE 20: note = X is Aib
  SITE 13: note = L is alpha- Methylleucine
HXQGTFTSDYSILLDKKAQXAFIEKLLKGGPSSGAPPPS

SEQ ID NO: 10 - protein, 39 aa, synthetic construct
  SITE 2: note = X is Aib
  SITE 20: note = X is Aib
  SITE 13: note = L is alpha- Methylleucine
YXQGTFTSDYSILLDKKYQXAFIEKLLKGGPSSGAPPPS

SEQ ID NO: 11 - protein, 39 aa, synthetic construct
  SITE 2: note = X is Aib
  SITE 20: note = X is Aib
  SITE 13: note = L is alpha- Methylleucine
YXQGTFTSDYSILLEKKAQXAFIEKLLKGGPSSGAPPPS

SEQ ID NO: 12 - protein, 39 aa, synthetic construct
  SITE 2: note = X is Aib
  SITE 20: note = X is Aib
HXHGTFTSDYSIYLEKKYAXEFVQELLKGGPSSGAPPPS

SEQ ID NO: 13 - protein, 39 aa, synthetic construct
  SITE 2: note = X is Aib
  SITE 20: note = X is Aib
  SITE 13: note = L is alpha- Methylleucine
YXQGTFTSDYSILLDKKAQXAFIEELLKGGPSSGAPPPS

SEQ ID NO: 14 - protein, 39 aa, synthetic construct
  SITE 2: note = X is Aib
  SITE 20: note = X is Aib
  SITE 13: note = L is alpha- Methylleucine
YXQGTFTSDYSILLDKKAQXAFIEWLLKGGPSSGAPPPS

SEQ ID NO: 15 - protein, 39 aa, synthetic construct
  SITE 2: note = X is Aib
  SITE 20: note = X is Aib
  SITE 13: note = L is alpha- Methylleucine
YXQGTFTSDYSILLDKKAQXKFIEFLLEGGPSSGAPPPS

SEQ ID NO: 16 - protein, 39 aa, synthetic construct
  SITE 2: note = X is Aib
  SITE 20: note = X is Aib
  SITE 13: note = L is alpha- Methylleucine
YXQGTFTSDYSILLDKKAQXEFIEYLLEGGPSSGAPPPS

SEQ ID NO: 17 - protein, 39 aa, synthetic construct
  SITE 2: note = X is Aib
  SITE 20: note = X is Aib
  SITE 13: note = L is alpha- Methylleucine
YXQGTFTSDYSILLDKKAQXAFIKYLLEGGPSSGAPPPS

SEQ ID NO: 18 - protein, 39 aa, synthetic construct; identical to SEQ ID NO: 1
  SITE 2: note = X is Aib
  SITE 20: note = X is Aib
  SITE 13: note = L is alpha- Methylleucine

SEQ ID NO: 19 - protein, 39 aa, synthetic construct
  SITE 2: note = X is Aib
  SITE 20: note = X is Aib
  SITE 13: note = L is alpha- Methylleucine
YXQGTFTSDYSILLDKKAKXAFIKYLLEGGPSSGAPPPS

SEQ ID NO: 20 - protein, 39 aa, synthetic construct
  SITE 2: note = X is Aib
  SITE 20: note = X is Aib
  SITE 13: note = L is alpha- Methylleucine
YXQGTFTSDYSILLDKKAQXKFIEYLLKGGPSSGAPPPS

SEQ ID NO: 21 - protein, 39 aa, synthetic construct
  SITE 2: note = X is Aib
  SITE 13: note = L is alpha- Methylleucine
  SITE 21: note = K is alpha- Methyllysine
YXQGTFTSDYSILLDKKAQAKFIEYLLEGGPSSGAPPPS

SEQ ID NO: 22 - protein, 39 aa, synthetic construct; identical to SEQ ID NO: 1
  SITE 2: note = X is Aib
  SITE 20: note = X is Aib
  SITE 13: note = L is alpha- Methylleucine
  SITE 21: note = K is D-lysine

SEQ ID NO: 23 - protein, 39 aa, synthetic construct
  SITE 2: note = X is Aib
  SITE 20: note = X is Aib
  SITE 13: note = L is alpha- Methylleucine
  SITE 21: note = X is L-Ornithine
YXQGTFTSDYSILLDKKAQXXFIEYLLEGGPSSGAPPPS

SEQ ID NO: 24 - protein, 39 aa, synthetic construct
  SITE 2: note = X is Aib
  SITE 20: note = X is Aib
  SITE 13: note = L is alpha- Methylleucine
YXQGTFTSDYSILKDKKAQXAFIEYLLEGGPSSGAPPPS

SEQ ID NO: 25 - protein, 39 aa, synthetic construct; identical to SEQ ID NO: 15
  SITE 2: note = X is Aib
  SITE 20: note = X is Aib
  SITE 13: note = L is alpha- Methylleucine

SEQ ID NO: 26 - protein, 39 aa, synthetic construct
  SITE 2: note = X is Aib
  SITE 20: note = X is Aib
  SITE 13: note = is alpha- Methylleucine
YXQGTFTSDYSILLDKKAQXKFIEFLIEGGPSSGAPPPS

SEQ ID NO: 27 - protein, 39 aa, synthetic construct
  SITE 2: note = X is Aib
  SITE 20: note = X is Aib
  SITE 13: note = L is alpha- Methylleucine
YXQGTFTSDYSILLDKKAQXKFVEFLIEGGPSSGAPPPS

SEQ ID NO: 28 - protein, 39 aa, synthetic construct
  SITE 2: note = X is Aib
  SITE 20: note = X is Aib
  SITE 13: note = L is alpha- Methylleucine
YXQGTFTSDYSILLDKKAQXAFIEKFIKGGPSSGAPPPS

SEQ ID NO: 29 - protein, 39 aa, synthetic construct
  SITE 2: note = X is Aib
  SITE 20: note = X is Aib
  SITE 13: note = L is alpha- Methylleucine
YXQGTFTSDYSILLDKKAQXKFIEFLLKGGPSSGAPPPS

SEQ ID NO: 30 - protein, 39 aa, synthetic construct
  SITE 2: note = X is Aib
  SITE 13: note = X is Aib
  SITE 20: note = X is Aib
YXQGTFTSDYSIXLDKKAQXKFIEFLLEGGPSSGAPPPS

SEQ ID NO: 31 - protein, 39 aa, synthetic construct
  SITE 2: note = X is Aib
  SITE 20: note = X is Aib
  SITE 13: note = L is alpha- Methylleucine
YXQGTFTSDYSKLLDKKAQXAFIEFLLEGGPSSGAPPPS

SEQ ID NO: 32 - protein, 39 aa, synthetic construct
  SITE 2: note = X is Aib
  SITE 20: note = X is Aib
  SITE 13: note = L is alpha- Methylleucine
YXQGTFTSDYSILLDKKAQXKFVEFLLKGGPSSGAPPPS

SEQ ID NO: 33 - protein, 39 aa, synthetic construct
  SITE 2: note = X is Aib
  SITE 20: note = X is Aib
  SITE 13: note = L is alpha- Methylleucine
YXQGTFTSDYSILLDKKAQXKFVEFLIKGGPSSGAPPPS

SEQ ID NO: 34 - protein, 39 aa, synthetic construct; identical to SEQ ID NO: 29
  SITE 2: note = X is Aib
  SITE 20: note = X is Aib
  SITE 13: note = L is alpha- Methylleucine

SEQ ID NO: 35 - protein, 39 aa, synthetic construct
  SITE 2: note = X is Aib
  SITE 20: note = X is Aib
  SITE 13: note = L is alpha- Methylleucine
YXQGTFTSDYSILLDKKAQXKFIKFLLEGGPSSGAPPPS

SEQ ID NO: 36 - protein, 39 aa, synthetic construct
  SITE 2: note = X is Aib
  SITE 20: note = X is Aib
  SITE 13: note = L is alpha- Methylleucine
YXQGTFTSDYSKLLDKKAQXKFIEFLLEGGPSSGAPPPS

SEQ ID NO: 37 - protein, 39 aa, synthetic construct
  SITE 2: note = X is Aib
  SITE 20: note = X is Aib
  SITE 13: note = L is alpha- Methylleucine
YXQGTFTSDYSILKDKKAQXEFIEYLLEGGPSSGAPPPS

SEQ ID NO: 38 - protein, 39 aa, synthetic construct
  SITE 2: note = X is Aib
  SITE 20: note = X is Aib
  SITE 13: note = L is alpha- Methylleucine
YXQGTFTSDYSILKDKKAQXAFIEYLLKGGPSSGAPPPS

SEQ ID NO: 39 - protein, 39 aa, synthetic construct
  SITE 2: note = X is Aib
  SITE 20: note = X is Aib
  SITE 13: note = L is alpha- Methylleucine
YXQGTFTSDYSILKDKKAQXAFIQYLLEGGPSSGAPPPS

SEQ ID NO: 40 - protein, 39 aa, synthetic construct
  SITE 2: note = X is Aib
  SITE 20: note = X is Aib
  SITE 13: note = L is alpha- Methylleucine
YXQGTFTSDYSILKDKKAQXKFIEYLLEGGPSSGAPPPS

SEQ ID NO: 41 - protein, 39 aa, synthetic construct
  SITE 2: note = X is Aib
  SITE 20: note = X is Aib
  SITE 13: note = L is alpha- Methylleucine
YXQGTFTSDYSILKDKKAQXLFIEYLLEGGPSSGAPPPS

SEQ ID NO: 42 - protein, 39 aa, synthetic construct; identical to SEQ ID NO: 24
  SITE 2: note = X is Aib
  SITE 20: note = X is Aib
  SITE 6: note = F is alpha- Methylphenylalanine
  SITE 13: note = L is alpha- Methylleucine

SEQ ID NO: 43 - protein, 39 aa, synthetic construct; identical to SEQ ID NO: 38
  SITE 2: note = X is Aib
  SITE 20: note = X is Aib
  SITE 13: note = L is alpha- Methylleucine
  SITE 6: note = F is alpha- Methylphenylalanine